European Patent Application EP 4 279 590 A1, published November 22, 2023. Title: sequencing. Applicant: Miltenyi Biotec BV & Co KG. The sequence listing filed with the application follows.

SEQUENCE LISTING (8 sequences)

SEQ ID NO: 1 - DNA, 12 bp, Artificial Sequence
  Oligo 1 of modified adapter
gatcggaagagc

SEQ ID NO: 2 - DNA, 34 bp, Artificial Sequence
  Oligo 2 of modified adapter
gtgactggagttcagacgtgtgctcttccgatct

SEQ ID NO: 3 - DNA, 49 bp, Artificial Sequence
  Target enrichment 1 forward primer (universal)
aatgatacggcgaccaccgagatctacactctttccctacacgacgctc

SEQ ID NO: 4 - DNA, 20 bp, Artificial Sequence
  Target enrichment 1 reverse primer (specific for TRA)
tgaaggcgtttgcacatgca

SEQ ID NO: 5 - DNA, 25 bp, Artificial Sequence
  Target enrichment 2 forward primer (universal)
aatgatacggcgaccaccgagatct

SEQ ID NO: 6 - DNA, 20 bp, Artificial Sequence
  Target enrichment 2 reverse primer (specific for TRA)
agtctctcagctggtacacg

SEQ ID NO: 7 - DNA, 20 bp, Artificial Sequence
  Target enrichment 1 reverse primer with modified base (specific for TRA)
  misc_feature (2)..(2): A is nucleotide analogue
taaaggcgtttgcacatgca

SEQ ID NO: 8 - DNA, 20 bp, Artificial Sequence
  Target enrichment 2 reverse primer with modified base (specific for TRA)
  misc_feature (2)..(2): A is nucleotide analogue
aatctctcagctggtacacg